European Patent Specification EP 3 612 207 B1, published April 10, 2024. Title: METHOD OF TREATMENT. Applicant: VOLUTION IMMUNO PHARMACEUTICALS SA. The sequence listing filed with the application follows.

SEQUENCE LISTING (19 sequences)

SEQ ID NO: 1 - DNA, 507 bp, Ornithodoros moubata
atgctggttttggtgaccctgattttctccttttctgcgaacatcgcatatgctgacagcgaaagcgactgcactggaagcgaacctgttgacgccttccaagctttcagtgagggcaaagaggcatatgtcctggtgaggtccacggatcccaaagcgagggactgcttgaaaggagaaccagccggagaaaagcaggacaacacgttgccggtgatgatgacgtttaagaatggcacagactgggcttcaaccgattggacgtttactttggacggcgcaaaggtaacggcaacccttggtaacctaacccaaaatagggaagtggtctacgactcgcaaagtcatcactgccacgttgacaaggtcgagaaggaagttccagattatgagatgtggatgctcgatgcgggagggcttgaagtggaagtcgagtgctgccgtcaaaagcttgaagagttggcgtctggcaggaaccaaatgtatccccatctcaaggactgctag

SEQ ID NO: 2 - protein, 168 aa, Ornithodoros moubata
MLVLVTLIFSFSANIAYADSESDCTGSEPVDAFQAFSEGKEAYVLVRSTDPKARDCLKGEPAGEKQDNTLPVMMTFKNGTDWASTDWTFTLDGAKVTATLGNLTQNREVVYDSQSHHCHVDKVEKEVPDYEMWMLDAGGLEVEVECCRQKLEELASGRNQMYPHLKDC

SEQ ID NO: 3 - protein, 150 aa, Ornithodoros moubata
DSESDCTGSEPVDAFQAFSEGKEAYVLVRSTDPKARDCLKGEPAGEKQDNTLPVMMTFKNGTDWASTDWTFTLDGAKVTATLGNLTQNREVVYDSQSHHCHVDKVEKEVPDYEMWMLDAGGLEVEVECCRQKLEELASGRNQMYPHLKDC

SEQ ID NO: 4 - DNA, 453 bp, Ornithodoros moubata
gacagcgaaagcgactgcactggaagcgaacctgttgacgccttccaagctttcagtgagggcaaagaggcatatgtcctggtgaggtccacggatcccaaagcgagggactgcttgaaaggagaaccagccggagaaaagcaggacaacacgttgccggtgatgatgacgtttaagaatggcacagactgggcttcaaccgattggacgtttactttggacggcgcaaaggtaacggcaacccttggtaacctaacccaaaatagggaagtggtctacgactcgcaaagtcatcactgccacgttgacaaggtcgagaaggaagttccagattatgagatgtggatgctcgatgcgggagggcttgaagtggaagtcgagtgctgccgtcaaaagcttgaagagttggcgtctggcaggaaccaaatgtatccccatctcaaggactgctag

SEQ ID NO: 5 - protein, 150 aa, Artificial Sequence
  Synthetic peptide
DSESDCTGSEPVDAFQAFSEGKEAYVLVRSTDPKARDCLKGEPAGEKQDNTLPVMMTFKNGTDWASTDWTFTLDGAKVTATLGNLTQNREVVYDSQSHHCHVDKVEKEVPDYEQWQSNGSADDKEVECCRQKLEELASGRNQMYPHLKDC

SEQ ID NO: 6 - protein, 150 aa, Artificial Sequence
  Synthetic peptide
DSESDCTGSEPVDAFQAFSEGKEAYVLVRSTDPKARDCLKGEPNGEKQDNTLPVMMTFKNGTDWASTDWTFTLDGAKVTATLGNLTQNREVVYDSQSHHCHVDKVEKEVPDYEMWQSDAGADAVEVECCRQKLEELASGRNQMYPHLKGC

SEQ ID NO: 7 - protein, 150 aa, Artificial Sequence
  Synthetic peptide
DSESDCTGSEPVDAFQAFSEGKEAYVLVRSTDPKARDCLKGEPNGEKQDNTLPVMMTFKNGTDWASTDWTFTLDGAKVTATLGNLTQNREVVYDSQSHHCHVDKVEKEVPDYEMWQLDAGGDEVEVECCRQKLEELASGRNQMYPHLKGC

SEQ ID NO: 8 - protein, 150 aa, Artificial Sequence
  Synthetic peptide
DSESDCTGSEPVDAFQAFSEGKEAYVLVRSTDPKARDCLKGEPNGEKQDNTLPVMMTFKNGTDWASTDWTFTLDGAKVTATLGNLTQNREVVYDSQSHHCHVDKVEKEVPDYEMWMLDAGGLEVEVECCRQKLEELASGRNQMYPHLKDC

SEQ ID NO: 9 - protein, 11 aa, Artificial Sequence
  Synthetic peptide
MWMLDAGGLEV

SEQ ID NO: 10 - protein, 11 aa, Artificial Sequence
  Synthetic peptide
QWQSNGSADDK

SEQ ID NO: 11 - protein, 11 aa, Artificial Sequence
  Synthetic peptide
MWQSDAGADAV

SEQ ID NO: 12 - protein, 11 aa, Artificial Sequence
  Synthetic peptide
MWQLDAGGDEV

SEQ ID NO: 13 - protein, 20 aa, Artificial Sequence
  PAS sequence
ASPAAPAPASPAAPAPSAPA

SEQ ID NO: 14 - protein, 20 aa, Artificial Sequence
  PAS sequence
AAPASPAPAAPSAPAPAAPS

SEQ ID NO: 15 - protein, 20 aa, Artificial Sequence
  PAS sequence
APSSPSPSAPSSPSPASPSS

SEQ ID NO: 16 - protein, 20 aa, Artificial Sequence
  PAS sequence
SAPSSPSPSAPSSPSPASPS

SEQ ID NO: 17 - protein, 20 aa, Artificial Sequence
  PAS sequence
SSPSAPSPSSPASPSPSSPA

SEQ ID NO: 18 - protein, 24 aa, Artificial Sequence
  PAS sequence
AASPAAPSAPPAAASPAAPSAPPA

SEQ ID NO: 19 - protein, 20 aa, Artificial Sequence
  PAS sequence
ASAAAPAAASAAASAPSAAA